European Patent Specification EP 3 560 951 B1, published February 14, 2024. Title: Generation of Haploid Plants and Improved Plant Breeding. Applicant: The Regents of the University of California. The sequence listing filed with the application follows.

SEQUENCE LISTING (114 sequences)

SEQ ID NO: 1 - protein, 136 aa, Arabidopsis thaliana
  thale cress histone 3.3 (H3.3), histone 3-like 1
MARTKQSARKSHGGKAPTKQLATKAARKSAPTTGGVKKPHRFRPGTVALREIRKYQKSTELLNRKLPFQRLVREIAQDFKTDLRFQSHAVLALQEAAEAYLVGLFEDTNLCAIHAKRVTIMPKDVQLARRIRAERA

SEQ ID NO: 2 - protein, 136 aa, Homo sapiens
  human histone 3.3 (H3.3), H3 histone, family 3A (H3F3A), H3 histone, family 3B (H3F3B)
MARTKQTARKSTGGKAPRKQLATKAARKSAPSTGGVKKPHRYRPGTVALREIRRYQKSTELLIRKLPFQRLVREIAQDFKTDLRFQSAAIGALQEASEAYLVGLFEDTNLCAIHAKRVTIMPKDIQLARRIRGERA

SEQ ID NO: 3 - protein, 125 aa, Physcomitrella patens
  moss histone H3
MARRKTTPVHGNHRASTSSVGGAAVRPRKPHRWRPGTKALQEIRHYQKTCDLLIPRLPFARYVKEITMMYASDVSRWTAEALTALQEATEDYMCHLFEDTNLCAIHAKRVTIMPKDLQLARRLRG

SEQ ID NO: 4 - protein, 164 aa, Pinus taeda
  loblolly pine histone H3
MVRRKTVPPRKKSGSGNAASTSGVGVSTPGSAGERGERRGSARLASTPGSDASPSAPSGRKPHRFRPGTVALREIKRYQKSFELLIPSLPFARIVRELTMYYSQVVSRWAAEALVALQEAAEDYIVHLFEDTNLCAIHAKRVTIMPRDLRLARRLRGGGLDRPW

SEQ ID NO: 5 - protein, 177 aa, Boechera holboellii
  Holboell's rockcress CENH3
MARTKHLATRSRPRNQTDATASSSQAAGPSTNPTTRGSEGEDAAQETTPTTSPATGRKKGAKRARYARPQGSQKKPYRYKPGTVALREIRYFQKSINLLIPAASFIRQVRSITHALAPPQITRWTAEALVALQEAAEDYLVGLFSDSMLCAIHARRVTLMRKDFELARRLGGKGRPW

SEQ ID NO: 6 - protein, 177 aa, Boechera stricta
  Drummond's rockcress CENH3
MARTKHLATRSRPRNWTDATASSSQAAGPTTNPTTRGSEGEDAAQEPTPTTSPATGRKKGAKRARYARPQGSQKKPYRYKPGTVALREIRHFQKSINLLIPAASFIRQVRSITHALAPPQITRWTAEALVALQEAAEDYLVGLFSDSMLCAIHARRITLMRKDFELARRLGGKGRPW

SEQ ID NO: 7 - protein, 180 aa, Lepidum virginicum
  Virginia pepperweed centromeric histone H3-like protein (CENH3)
MARTKRYASRPQRPRNQTDVTVPSSPAAGPSTNPTRRDSEGEGGDDAQQTVPTTSPASISKKASKKNRKATPQSSKKKTYRYKPGTVALREIRHFQKSTHLLIPAAAFIREVRCITQAVAPPQISRWTAEALVALQEAAEDYVVGLLSDSMLCAIHARRVTLMRKDFELARRLGGKGRPW

SEQ ID NO: 8 - protein, 172 aa, Cardamine flexuosa
  woodland bittercress centromeric histone H3-like protein (CENH3)
MARTKHFPNRTRPRNQTDATTPAAGPSTRTTRANQGEETQQTNPTTSPATSKKKGAKRTRRDMPQGSQKKPYRYKPGTVALREIRHFQKSTNLLIPAASFIRQVRSITQMYAPPQINRWTAEALVALQEAAEDYLVGLFSDSMLCAIHARRVTLMRKDFELARRLGGKGRPW

SEQ ID NO: 9 - protein, 139 aa, Hordeum vulgare
  barley CENH3
MARTKKTVAAKEKRPPCSKSEPQSQPKKKEKRAYRFRPGTVALREIRKYRKSTNMLIPFAPFVRLVRDIADNLTPLSNKKESKPTPWTPLALLSLQESAEYHLVDLFGKANLCAIHSHRVTIMLKDMQLARRIGTRSLW

SEQ ID NO: 10 - protein, 178 aa, Arabidopsis thaliana
  thale cress histone H3-like centromere protein (CENH3)
MARTKHRVTRSQPRNQTDAAGASSSQAAGPTTTPTRRGGEGGDNTQQTNPTTSPATGTRRGAKRSRQAMPRGSQKKSYRYRPGTVALKEIRHFQKQTNLLIPAASFIREVRSITHMLAPPQINRWTAEALVALQEAAEDYLVGLFSDSMLCAIHARRVTLMRKDFELARRLGGKGRPW

SEQ ID NO: 11 - protein, 152 aa, Populus trichocarpa
  black cottonwood histone H3
MARTKHPVARKRARSPKRSDASPSTPRTPTSSRTRPQANGQQGSSTQRQRKKHRFRSGTVALREIRQYQKTWRPLIPAASFIRCVRMITQEFSREVNRWTAEALVAIQEAAEDFLVHLFEDGMLCAIHAKRVTLMKKDFELARRLGGKGRPW

SEQ ID NO: 12 - protein, 166 aa, Triticum aestivum
  wheat CENH3
MARTKHPAVRKTKALPKKQLGTRPSAGTPRRQETDGAGTSATPRRAGRAAAPGAAEGATGQPKQRKPHRFRPGTVALREIRKYQKSVDFLIPFAPFVRLIKEVTDFFCPEISRWTPQALVAIQEAAEYHLVDVFERANHCAIHAKRVTVMQKDIQLARRIGGRRLW

SEQ ID NO: 13 - protein, 170 aa, Oryza sativa
  rice centromeric histone 3 (CENH3)
MARTKHPAVRKSKAEPKKKLQFERSPRPSKAQRAGGGTGTSATTRSAAGTSASGTPRQQTKQRKPHRFRPGTVALREIRKFQKTTELLIPFAPFSRLVREITDFYSKDVSRWTLEALLALQEAAEYHLVDIFEVSNLCAIHAKRVTIMQKDMQLARRIGGRRPWNLNSLR

SEQ ID NO: 14 - protein, 167 aa, Luzula nivea
  snowy woodrush centromere specific histone H3 variant (CENH3)
MARTKHFPQCSRHPKKQRTAAGEAGSSVIAKQNAPAKTGNASSITNSTPARSLKKNKASKRGEKTQAKQRKMYRYRPGTVALREIRKLQKTTDLLVPKASFARLVKEITFQSSKEVNRWQAEALIALQEASECFLVNLLESANMLAIHARRVTIMKKDIQLARRIGA

SEQ ID NO: 15 - protein, 176 aa, Arabidopsis arenosa
  sand rockcress CENH3
MARTKHFATRTGSGNRTDANASSSQAAGPTTTPTTRGTEGGDNTQQTNPTTSPATGGRRPRRARQAMPRGSQKKPYRYKPGTVALREIRHFQKQTNLLIPAASFIRQVRSITHALAPPQINRWTAEALVALQEAAEDYLIGLFSDSMLCAIHARRVTLMRKDFELARRLGGKGRPW

SEQ ID NO: 16 - protein, 157 aa, Zea mays
  corn centromeric histone H3 (CENH3)
MARTKHQAVRKTAEKPKKKLQFERSGGASTSATPERAAGTGGRAASGGDSVKKTKPRHRWRPGTVALREIRKYQKSTEPLIPFAPFVRVVRELTNFVTNGKVERYTAEALLALQEAAEFHLIELFEMANLCAIHAKRVTIMQKDIQLARRIGGRRWA

SEQ ID NO: 17 - protein, 154 aa, Sorghum bicolor
  sorghum CENH3
MARTKHQAVRKLPQKPKKKLQFERAGGASTSATPRRNAGTGGGAAARGEDLFKKHRWRAGTVALREIRKYQKSTEPLIPFAPFVRVVKELTAFITDWRIGRYTPEALLALQEAAEFHLIELFEVANLCAIHAKRVTVMQKDIQLARRIGGRRWS

SEQ ID NO: 18 - protein, 150 aa, Cichorium intybus
  chicory CENH3
MARTKQPAKRSWGNRKSSQSRASTSTSTSTPRKSPRKDPGRTGERRQQKPHRFKPGAQALREIRRLQKTVNLLIPAAPFIRTVKEISNYIAPEVTRWQAEAIQALQEAAEDYLVQLFEDSMLCSIHAKRVTLMKKDWELARRLTKKGQPW

SEQ ID NO: 19 - protein, 153 aa, Cycas rumphii
  queen sago CENH3
MARKKASTPRKKTGTAASTSAVESPPSGVNQTARARRSVGGVAPGAPRTPQASTNVGTPRRPHRFRPGTVALREIRRYQKSFELLIPALPFARNVRELTLHHSREVHRWTAEALVALQEAAEDYIVHLFEDTNLCAIHAKRVTIMPKDMHLAR

SEQ ID NO: 20 - protein, 154 aa, Allium cepa
  onion CENH3
MARTKQMAHKKLRRKLNVDEAGPSTPVTRSTEVNPKSSRPTPITEDRGTGARKKHRFRPGTVALREIRKYQKTAELLIPAAPFIRLVREITNLYSKEVTRWTPEALLAIQEAAEFFIINLLEEANLCAIHAKRVTLMQKDIQLARRIGGARHFS

SEQ ID NO: 21 - protein, 199 aa, Malus domestica
  apple CENH3
MARIKHTAHKKSVARKSSTPKEAAAGTGGTSAASPAKQPEPSAPWRRSERSSQRTSESQEQQEPETNAQATPQSKKQKQSERNPQTPQSKKQKPSERNPPPTQKKKWRYRPGTVALREIRYYQKTWNLIIPAAPFIRTVREISINMSKDPVRWTPEALQAIQEAAEDFLVRLFEDSMLCAIHARRVTLMKKDLELARRI

SEQ ID NO: 22 - protein, 150 aa, Lactuca sativa
  lettuce CENH3
MARTKQPAKRSWGKRQSAGASTSTSTSTPRKSPRKDPGSSGTGQRQKQKPHRFKPGTQALREIRRLQKTVNLLIPAAPFIRTVKEISNYIAPEVTRWQAEALQALQEAAEDYIVQLFEDSMLCSIHAKRVTLMKKDMELARRLTKKGQPW

SEQ ID NO: 23 - protein, 145 aa, Carthamus tinctorius
  safflower CENH3
MARTKQPAKRSSGKRDARPSTSTPTPRPSARKNPESSGAGDGQRRHRYRPGTQALREIRRLQKTVNLLIPAAPFIRTVKEISNYIAPEVTRWQAEALQALQEAAEDYLIQLFEDSMLCAIHAKRVTLMKKDWELARRLGKKGQPW

SEQ ID NO: 24 - protein, 142 aa, Helianthus exilis
  serpentine sunflower CENH3
MARTKHPAKRSSGIPVDGRSSTSTNTPRKSPRKNRGGENRKPHRFKPGTQALREIRRLQKTVELIIPAAPFIRTVKEISNYMAPEITRWQAEALQALQEAAEDYLIQLFEDSMLCAIHAKRVTLMKKDWELARRIGKKGQPW

SEQ ID NO: 25 - protein, 152 aa, Gossypium hirsutum
  upland cotton CENH3
MSRTKHTAAKKPRRKPSAAAAASPATASPHTRSVTAKKTGGPATPTPGKSKRPHRFRAGTRALQEIRKYQKTSNLLVPAASFIREVRAISYRFAPDINRWQAEALVAIQEAEDYLIQLFGDAMLCAIHAKRVTLMKKDIQLARRLGGMGQPW

SEQ ID NO: 26 - protein, 155 aa, Glycine max
  soybean CENH3
MARVKHTPASRKSAKKQAPRASTSTQPPPQSQSPATRERRRAQQVEPQQEPEAQGRKKRRNRSGTVALREIRHFQRSCELLIPAAPFIRCVKQITNQFSTEVSRWTPEAVVALQEAAEEYLVHLFEDGMLCAIHARRITLMKKDIELARRLGGIG

SEQ ID NO: 27 - protein, 153 aa, Cucumis melo
  cantaloupe CENH3
MARARHPVQRKSNRTSSGSGAALSPPAVPSTPLNGRTQNVRKAQSPPSRTKKKIRFRPGTVALREIRNLQKSWNLLIPASCFIRAVKEVSNQLAPQITRWQAEALVALQEAAEDFLVHLFEDTMLCAIHAKRVTIMKKDFELARRLGGKGRPW

SEQ ID NO: 28 - protein, 147 aa, Solanum chacoense
  Chaco potato CENH3
MARTKHLAKRSRTKPSVAAGPSATPSTPTRKSPRSAPATSVPKPKQKKRYRPGSVALREIRHFQKTWNLVIPAAPFIRLVREISHFFAPGVTRWQAEALIAIQEAAEDFLVHLFEDAMLCAIHAKRVTLMKKDFELARRLGGKGQPW

SEQ ID NO: 29 - protein, 144 aa, Solanum lycopersicum
  tomato CENH3
MARTKHLAKRSRTTSAAPSATPSTPSRKSPRSAPATSVQKPKQKKRYRPGTVALREIRHFQKTWDLLIPAAPFIRLVREISHFYAPGVTRWQAEALIAIQEAAEDFLVHLFEDAMLCAIHAKRVTLMKKDFELARRLGGKGQPW

SEQ ID NO: 30 - protein, 156 aa, Nicotiana tabacum
  allotetraploid tobacco centromere specific histone H3 variant (CENH3-1)
MARTKHLALRKQSRPPSRPTATRSAAAAASSAPQSTPTRTSQRTAPSTPGRTQKKKTRYRPGTVALREIRRFQKTWDLLIPAAPFIRLVKEISHFFAPEVTRWQAEALIALQEAAEDFLVHLFDDSMLCAIHAKRVTLMKKDFELARRLGGKARPW

SEQ ID NO: 31 - protein, 157 aa, Nicotiana tabacum
  allotetraploid tobacco centromere specific histone H3 variant (CENH3-2)
MARTKHLALRKQSRPPSRPTATRSAAAAASSSAPQSTPTRTSQRTAPSTPGRTQKKKTRYRPGTVALREIRRFQKTWNLLIPAAPFIRLVKEISYFFAPEVTRWQAEALIALQEAAEDFLVHLFDDSMLCAIHAKRVTLMKKDFELARRLGGKARPW

SEQ ID NO: 32 - protein, 156 aa, Nicotiana tomentosiformis; identical to SEQ ID NO: 30
  diploid tobacco centromere specific histone H3 variant (CENH3)

SEQ ID NO: 33 - protein, 158 aa, Vitis vinifera
  European wine grape CENH3
MTRTKHLARKSRNRRRQFAATPASPASAGPSSAPPRRPTRTATDASPSTAGSQGQRKPFRYRPGTVALREIRRFQKTTHLLIPAAPFIRTVREISYFFAPEISRWTAEALVALQEAAEDYLVHLFEDAMLCAIHAKRVTLMKKDWELARRIGGKGQPW

SEQ ID NO: 34 - protein, 157 aa, Nicotiana sylvestris; identical to SEQ ID NO: 31
  woodland tobacco centromere specific histone H3 variant (CENH3)

SEQ ID NO: 35 - protein, 177 aa, Crucihimalaya himalaica
  Himalayan rockcress centromeric histone (CENH3)
MARTKHFATRSRPRNQTDATASASQATGPSTNPTTRGSEGEDAARGTNPTTSPATGRKKGVKRARHAMPQGSQKKPYRYKAGTVALREIRHFQKNTNLLIPAASFIRQVKSITYAVAPPQITRWTAEALVALQEAAEDYLVGLFSDSMLCAIHARRVTLMRKDFELARRLGGKGRPW

SEQ ID NO: 36 - protein, 176 aa, Arabidopsis lyrata
  lyre-leaved rockcress centromeric histone (CENH3)
MARTKHFATKSRSGNRTDANASSSQAAGPTTTPTTRGTEGGDNTQQTNPTTSPATGGRRPRRARQAMPRVSQNKPYRYKPGTVALREIRHFQKQTNLLIPAASFIRQVRSITHALAPPQINRWTAEALVALQEAAEDYLVGLFSDSMLCAIHARRVTLMRKDFELARRLGGKGRPW

SEQ ID NO: 37 - protein, 170 aa, Capsella bursapastoris
  shepherd's purse centromeric histone (CENH3)
MARTKHFATRSGPRTPAVASSSQAAVPSSSPATRGRVGVDAAAQQPTPATSPATAKKKGAKRARFGRPQGSQKKKPYRYRPGTVALREIRHYQKGTSLLIPAAAFIRQVRSITNAVAPREVNRWTAEALVALQEAAEDFLVGLFSDSMLCAIHARRVTLMRKDFDLARRL

SEQ ID NO: 38 - protein, 178 aa, Raphanus sativus
  radish centromeric histone H3-like protein (CENH3)
MARTKHFASRARDRNQPNAAAAAAGPSATPTRRGSSQGEEAQQTTPTTTSPATTASGRKKGTKRTTQAMPKSSKKKTFRYKPGTVALREIRHFQKSTKLLIPSAPFIREVRSITHNLAAAYVTRWTAEALIALQEAAEDFLVGLFSDAMLCAIHAKRVTLMRKDFELARRLGGKGRPF

SEQ ID NO: 39 - protein, 164 aa, Eruca sativa
  arugula centromeric histone H3-like protein (CENH3)
MARTKHFASRARDRNRNNATASSSAAAAAAGPSATPTRRGSRQGGGGGGGVEAQQGSNKKKKSFRYKPGTVALREIRHFQKTTKLLIPAATFIRLVRSITLDRAKPQVTRWTAEALVALQEAAEDYLVGLFSDSMLCAIHAKRVTLMRKDFELARRLGGKGRPW

SEQ ID NO: 40 - protein, 173 aa, Olimarabidopsis pumila
  dwarf rocket centromeric histone H3-like protein 1 (CENH3-1)
MARTKHNAIRSRDRTGATASSSQAAGPSTNPTAGGSEDAAQQTTPTTSPATGSKKRAKRARQAMPRGSQKKPYRYKPGTVALREIRHFQKTTSLLLPAAPFIRQVRSISSALAPREITRWTAEALVALQEAAEDYLVGLFSDSMLCAIHAKRVTLMRKDFELARRLGGKGRPW

SEQ ID NO: 41 - protein, 174 aa, Olimarabidopsis pumila
  dwarf rocket centromeric histone H3-like protein 2 (CENH3-2)
MTRTKHTVIKSSRPLDRTDASSSQAAGPSTNPTAGSSGDAAQQTTPTTSPATGSTKRAKRARQAMPRGSQKKPYRYKPGTVALREIRHFQKTTSFLIPAAPFIRQVRSISSALAPTQITRWTAEALVALQEAAEDYLVGLFSDSMLCAIHAKRVTLMRKDFELARRLGGKGRPW

SEQ ID NO: 42 - protein, 174 aa, Turritis glabra
  tower mustard histone H3 like protein (CENH3)
MARTKHFATRSRPRNQTDSSSQAAGPSTNPTTGGSEGGDAAQQTTPTTSPATGRKKRAKRAKQAMPQGSQKKPYRYKPGTIALREIRYFQKNTNLLIPAASFIREVRSITHALAPPQISRWTAEALVALQEAAEDYLVGLFSDSMLCAIHARRVTLMRKDFELARRIGGKGRPW

SEQ ID NO: 43 - protein, 176 aa, Arabidopsis halleri
  histone H3 like protein 1 (CENH3-1)
MARTKHFAIKSRSGNRTDANASSSQAAGPTTTPTTRGTEGGDNTQQTNPTTSPATGGRRPRRARQAMPRGSQKKPYRYKPGTVALREIRHFQKQTNLLIPAASFIRQVRSITHALAPPQINRWTAEALVALQEAAEDYLVGLFSDSMLCAIHARRVTLMRKDFELTRRLGGKGRPW

SEQ ID NO: 44 - protein, 176 aa, Arabidopsis halleri
  histone H3 like protein 2 (CENH3-2)
MARTKHFVTRKGSGNRTDFDANASSSQAAGPTKTPTTRGTEGGDNTQQTTSPATGGRRGPRRARQAMPRGSQKKPYRYKPGTVALREIRHFQKQTNLLIPAASFIRQVRSITHALAPPQINRWTAEALVALQEAAEDYLVGLFSDSMLCAIHARRVTLMRKDFELARRLGGKGRPW

SEQ ID NO: 45 - protein, 175 aa, Arabidopsis lyrata
  lyre-leaved rockcress histone H3 (HTR12A)
MARTKHFATRTGSGNRTDANASSSSQAAGPTKTPTTRGTEGGDNTQQTTSPATGGRRGPRRARQAMPRGSQKKPYRYKPGTVALREIRHFQKQTNLLIPAASFIRQARSITHALAPPQINRWTAEALVALQEAAEDYLVGLFSDSMLCAIHARRVTLMRKDFELARRLGGKGRPW

SEQ ID NO: 46 - protein, 172 aa, Arabidopsis lyrata
  lyre-leaved rockcress histone H3 (HTR12B)
MARTKHFATKSRTDANASSSQAAGPTTTPTTRGTEGGDNTQQTNPTTSPATGGRRPRRARQAMPRGSQKKPYRYKPGTVALREIRHFQKQTNLLIPAASFIRQVRSITHALAPPQINRWTAEALVALQEAAEDYLVGLFSDSMLCAIHARRVTLMRKDFELARRLGGKGRPW

SEQ ID NO: 47 - protein, 163 aa, Saccharum officinalis
  sugarcane CENH3
MARTKHQAVRRPTQKPKKKLQFERAGGASTSATPERNAGTGGGAAARVTRGRVEKKHRWRVGTVALREIRKYQKSTEPLIPFAPFVRVVKELTGFITDWRIGRYTPEALLALQEAAEFHLIELFQVANLCAIHAKRVTVMQKDIQLARRIGGKRWAYPFFLPY

SEQ ID NO: 48 - protein, 181 aa, Brassica napa
  turnip CENH3
MARTKHFASRARDRNPTNATASSSAAAAAGPSATPTRRGGSQGGEAQQTTPPATTTAGRKKGGTKRTKQAMPKSSNKKKTFRYKPGTVALREIRHFQKTTKLLIPAASFIREVRSVTQIFAPPDVTRWTAEALMAIQEAAEDFLVGLFSDAMLCAIHARRVTLMRKDFELARRLGGKGRPL

SEQ ID NO: 49 - protein, 91 aa, Artificial Sequence
  Physcomitrella patens moss CENH3 histone domain
PGTKALQEIRHYQKTCDLLIPRLPFARYVKEITMMYASDVSRWTAEALTALQEATEDYMCHLFEDTNLCAIHAKRVTIMPKDLQLARRLRG

SEQ ID NO: 50 - protein, 98 aa, Artificial Sequence
  Pinus taeda loblolly pine CENH3 histone domain
PGTVALREIKRYQKSFELLIPSLPFARIVRELTMYYSQVVSRWAAEALVALQEAAEDYIVHLFEDTNLCAIHAKRVTIMPRDLRLARRLRGGGLDRPW

SEQ ID NO: 51 - protein, 97 aa, Artificial Sequence
  Boechera holboellii Holboell's rockcress CENH3 histone domain
PGTVALREIRYFQKSINLLIPAASFIRQVRSITHALAPPQITRWTAEALVALQEAAEDYLVGLFSDSMLCAIHARRVTLMRKDFELARRLGGKGRPW

SEQ ID NO: 52 - protein, 97 aa, Artificial Sequence
  Boechera stricta Drummond's rockcress CENH3 histone domain
PGTVALREIRHFQKSINLLIPAASFIRQVRSITHALAPPQITRWTAEALVALQEAAEDYLVGLFSDSMLCAIHARRITLMRKDFELARRLGGKGRPW

SEQ ID NO: 53 - protein, 97 aa, Artificial Sequence
  Lepidum virginicum Virginia pepperweed CENH3 histone domain
PGTVALREIRHFQKSTHLLIPAAAFIREVRCITQAVAPPQISRWTAEALVALQEAAEDYVVGLLSDSMLCAIHARRVTLMRKDFELARRLGGKGRPW

SEQ ID NO: 54 - protein, 97 aa, Artificial Sequence
  Cardamine flexuosa woodland bittercress CENH3 histone domain
PGTVALREIRHFQKSTNLLIPAASFIRQVRSITQMYAPPQINRWTAEALVALQEAAEDYLVGLFSDSMLCAIHARRVTLMRKDFELARRLGGKGRPW

SEQ ID NO: 55 - protein, 102 aa, Artificial Sequence
  Hordeum vulgare barley CENH3 histone domain
PGTVALREIRKYRKSTNMLIPFAPFVRLVRDIADNLTPLSNKKESKPTPWTPLALLSLQESAEYHLVDLFGKANLCAIHSHRVTIMLKDMQLARRIGTRSLW

SEQ ID NO: 56 - protein, 97 aa, Artificial Sequence
  Arabidopsis thaliana thale cress CENH3 histone domain
PGTVALKEIRHFQKQTNLLIPAASFIREVRSITHMLAPPQINRWTAEALVALQEAAEDYLVGLFSDSMLCAIHARRVTLMRKDFELARRLGGKGRPW

SEQ ID NO: 57 - protein, 96 aa, Artificial Sequence
  Populus trichocarpa black cottonwood CENH3 histone domain
SGTVALREIRQYQKTWRPLIPAASFIRCVRMITQEFSREVNRWTAEALVAIQEAAEDFLVHLFEDGMLCAIHAKRVTLMKKDFELARRLGGKGRPW

SEQ ID NO: 58 - protein, 95 aa, Artificial Sequence
  Triticum aestivum wheat CENH3 histone domain
PGTVALREIRKYQKSVDFLIPFAPFVRLIKEVTDFFCPEISRWTPQALVAIQEAAEYHLVDVFERANHCAIHAKRVTVMQKDIQLARRIGGRRLW

SEQ ID NO: 59 - protein, 101 aa, Artificial Sequence
  Oryza sativa rice CENH3 histone domain
PGTVALREIRKFQKTTELLIPFAPFSRLVREITDFYSKDVSRWTLEALLALQEAAEYHLVDIFEVSNLCAIHAKRVTIMQKDMQLARRIGGRRPWNLNSLR

SEQ ID NO: 60 - protein, 91 aa, Artificial Sequence
  Luzula nivea snowy woodrush CENH3 histone domain
PGTVALREIRKLQKTTDLLVPKASFARLVKEITFQSSKEVNRWQAEALIALQEASECFLVNLLESANMLAIHARRVTIMKKDIQLARRIGA

SEQ ID NO: 61 - protein, 97 aa, Artificial Sequence
  Arabidopsis arenosa sand rockcress CENH3 histone domain
PGTVALREIRHFQKQTNLLIPAASFIRQVRSITHALAPPQINRWTAEALVALQEAAEDYLIGLFSDSMLCAIHARRVTLMRKDFELARRLGGKGRPW

SEQ ID NO: 62 - protein, 96 aa, Artificial Sequence
  Zea mays corn CENH3 histone domain
PGTVALREIRKYQKSTEPLIPFAPFVRVVRELTNFVTNGKVERYTAEALLALQEAAEFHLIELFEMANLCAIHAKRVTIMQKDIQLARRIGGRRWA

SEQ ID NO: 63 - protein, 96 aa, Artificial Sequence
  Sorghum bicolor sorghum CENH3 histone domain
AGTVALREIRKYQKSTEPLIPFAPFVRVVKELTAFITDWRIGRYTPEALLALQEAAEFHLIELFEVANLCAIHAKRVTVMQKDIQLARRIGGRRWS

SEQ ID NO: 64 - protein, 96 aa, Artificial Sequence
  Cichorium intybus chicory CENH3 histone domain
PGAQALREIRRLQKTVNLLIPAAPFIRTVKEISNYIAPEVTRWQAEAIQALQEAAEDYLVQLFEDSMLCSIHAKRVTLMKKDWELARRLTKKGQPW

SEQ ID NO: 65 - protein, 87 aa, Artificial Sequence
  Cycas rumphii queen sago CENH3 histone domain
PGTVALREIRRYQKSFELLIPALPFARNVRELTLHHSREVHRWTAEALVALQEAAEDYIVHLFEDTNLCAIHAKRVTIMPKDMHLAR

SEQ ID NO: 66 - protein, 96 aa, Artificial Sequence
  Allium cepa onion CENH3 histone domain
PGTVALREIRKYQKTAELLIPAAPFIRLVREITNLYSKEVTRWTPEALLAIQEAAEFFIINLLEEANLCAIHAKRVTLMQKDIQLARRIGGARHFS

SEQ ID NO: 67 - protein, 89 aa, Artificial Sequence
  Malus domestica apple CENH3 histone domain
PGTVALREIRYYQKTWNLIIPAAPFIRTVREISINMSKDPVRWTPEALQAIQEAAEDFLVRLFEDSMLCAIHARRVTLMKKDLELARRI

SEQ ID NO: 68 - protein, 96 aa, Artificial Sequence
  Lactuca sativa lettuce CENH3 histone domain
PGTQALREIRRLQKTVNLLIPAAPFIRTVKEISNYIAPEVTRWQAEALQALQEAAEDYIVQLFEDSMLCSIHAKRVTLMKKDMELARRLTKKGQPW

SEQ ID NO: 69 - protein, 96 aa, Artificial Sequence
  Carthamus tinctorius safflower CENH3 histone domain
PGTQALREIRRLQKTVNLLIPAAPFIRTVKEISNYIAPEVTRWQAEALQALQEAAEDYLIQLFEDSMLCAIHAKRVTLMKKDWELARRLGKKGQPW

SEQ ID NO: 70 - protein, 96 aa, Artificial Sequence
  Helianthus exilis serpentine sunflower CENH3 histone domain
PGTQALREIRRLQKTVELIIPAAPFIRTVKEISNYMAPEITRWQAEALQALQEAAEDYLIQLFEDSMLCAIHAKRVTLMKKDWELARRIGKKGQPW

SEQ ID NO: 71 - protein, 95 aa, Artificial Sequence
  Gossypium hirsutum upland cotton CENH3 histone domain
AGTRALQEIRKYQKTSNLLVPAASFIREVRAISYRFAPDINRWQAEALVAIQEAEDYLIQLFGDAMLCAIHAKRVTLMKKDIQLARRLGGMGQPW

SEQ ID NO: 72 - protein, 93 aa, Artificial Sequence
  Glycine max soybean CENH3 histone domain
SGTVALREIRHFQRSCELLIPAAPFIRCVKQITNQFSTEVSRWTPEAVVALQEAAEEYLVHLFEDGMLCAIHARRITLMKKDIELARRLGGIG

SEQ ID NO: 73 - protein, 96 aa, Artificial Sequence
  Cucumis melo cantaloupe CENH3 histone domain
PGTVALREIRNLQKSWNLLIPASCFIRAVKEVSNQLAPQITRWQAEALVALQEAAEDFLVHLFEDTMLCAIHAKRVTIMKKDFELARRLGGKGRPW

SEQ ID NO: 74 - protein, 96 aa, Artificial Sequence
  Solanum chacoense Chaco potato CENH3 histone domain
PGSVALREIRHFQKTWNLVIPAAPFIRLVREISHFFAPGVTRWQAEALIAIQEAAEDFLVHLFEDAMLCAIHAKRVTLMKKDFELARRLGGKGQPW

SEQ ID NO: 75 - protein, 96 aa, Artificial Sequence
  Solanum lycopersicum tomato CENH3 histone domain
PGTVALREIRHFQKTWDLLIPAAPFIRLVREISHFYAPGVTRWQAEALIAIQEAAEDFLVHLFEDAMLCAIHAKRVTLMKKDFELARRLGGKGQPW

SEQ ID NO: 76 - protein, 96 aa, Artificial Sequence
  Nicotiana tabacum allotetraploid tobacco CENH3-1 histone domain
PGTVALREIRRFQKTWDLLIPAAPFIRLVKEISHFFAPEVTRWQAEALIALQEAAEDFLVHLFDDSMLCAIHAKRVTLMKKDFELARRLGGKARPW

SEQ ID NO: 77 - protein, 96 aa, Artificial Sequence
  Nicotiana tabacum allotetraploid tobacco CENH3-2 histone domain
PGTVALREIRRFQKTWNLLIPAAPFIRLVKEISYFFAPEVTRWQAEALIALQEAAEDFLVHLFDDSMLCAIHAKRVTLMKKDFELARRLGGKARPW

SEQ ID NO: 78 - protein, 96 aa, Artificial Sequence; identical to SEQ ID NO: 76
  Nicotiana tomentosiformis diploid tobacco CENH3 histone domain

SEQ ID NO: 79 - protein, 96 aa, Artificial Sequence
  Vitis vinifera European wine grape CENH3 histone domain
PGTVALREIRRFQKTTHLLIPAAPFIRTVREISYFFAPEISRWTAEALVALQEAAEDYLVHLFEDAMLCAIHAKRVTLMKKDWELARRIGGKGQPW

SEQ ID NO: 80 - protein, 96 aa, Artificial Sequence; identical to SEQ ID NO: 77
  Nicotiana sylvestris woodland tobacco CENH3 histone domain

SEQ ID NO: 81 - protein, 97 aa, Artificial Sequence
  Crucihimalaya himalaica Himalayan rockcress CENH3 histone domain
AGTVALREIRHFQKNTNLLIPAASFIRQVKSITYAVAPPQITRWTAEALVALQEAAEDYLVGLFSDSMLCAIHARRVTLMRKDFELARRLGGKGRPW

SEQ ID NO: 82 - protein, 97 aa, Artificial Sequence
  Arabidopsis lyrata lyre-leaved rockcress CENH3 histone domain
PGTVALREIRHFQKQTNLLIPAASFIRQVRSITHALAPPQINRWTAEALVALQEAAEDYLVGLFSDSMLCAIHARRVTLMRKDFELARRLGGKGRPW

SEQ ID NO: 83 - protein, 90 aa, Artificial Sequence
  Capsella bursapastoris shepherd's purse CENH3 histone domain
PGTVALREIRHYQKGTSLLIPAAAFIRQVRSITNAVAPREVNRWTAEALVALQEAAEDFLVGLFSDSMLCAIHARRVTLMRKDFDLARRL

SEQ ID NO: 84 - protein, 97 aa, Artificial Sequence
  Raphanus sativus radish CENH3 histone domain
PGTVALREIRHFQKSTKLLIPSAPFIREVRSITHNLAAAYVTRWTAEALIALQEAAEDFLVGLFSDAMLCAIHAKRVTLMRKDFELARRLGGKGRPF

SEQ ID NO: 85 - protein, 97 aa, Artificial Sequence
  Eruca sativa arugula CENH3 histone domain
PGTVALREIRHFQKTTKLLIPAATFIRLVRSITLDRAKPQVTRWTAEALVALQEAAEDYLVGLFSDSMLCAIHAKRVTLMRKDFELARRLGGKGRPW

SEQ ID NO: 86 - protein, 97 aa, Artificial Sequence
  Olimarabidopsis pumila dwarf rocket CENH3-1 histone domain
PGTVALREIRHFQKTTSLLLPAAPFIRQVRSISSALAPREITRWTAEALVALQEAAEDYLVGLFSDSMLCAIHAKRVTLMRKDFELARRLGGKGRPW

SEQ ID NO: 87 - protein, 97 aa, Artificial Sequence
  Olimarabidopsis pumila dwarf rocket CENH3-2 histone domain
PGTVALREIRHFQKTTSFLIPAAPFIRQVRSISSALAPTQITRWTAEALVALQEAAEDYLVGLFSDSMLCAIHAKRVTLMRKDFELARRLGGKGRPW

SEQ ID NO: 88 - protein, 97 aa, Artificial Sequence
  Turritis glabra tower mustard CENH3 histone domain
PGTIALREIRYFQKNTNLLIPAASFIREVRSITHALAPPQISRWTAEALVALQEAAEDYLVGLFSDSMLCAIHARRVTLMRKDFELARRIGGKGRPW

SEQ ID NO: 89 - protein, 97 aa, Artificial Sequence
  Arabidopsis halleri CENH3-1 histone domain
PGTVALREIRHFQKQTNLLIPAASFIRQVRSITHALAPPQINRWTAEALVALQEAAEDYLVGLFSDSMLCAIHARRVTLMRKDFELTRRLGGKGRPW

SEQ ID NO: 90 - protein, 97 aa, Artificial Sequence; identical to SEQ ID NO: 82
  Arabidopsis halleri CENH3-2 histone domain

SEQ ID NO: 91 - protein, 97 aa, Artificial Sequence
  Arabidopsis lyrata CENH3 HTR12A histone domain
PGTVALREIRHFQKQTNLLIPAASFIRQARSITHALAPPQINRWTAEALVALQEAAEDYLVGLFSDSMLCAIHARRVTLMRKDFELARRLGGKGRPW

SEQ ID NO: 92 - protein, 97 aa, Artificial Sequence; identical to SEQ ID NO: 82
  Arabidopsis lyrata CENH3 HTR12B histone domain

SEQ ID NO: 93 - protein, 103 aa, Artificial Sequence
  Saccharum officinalis sugarcane CENH3 histone domain
VGTVALREIRKYQKSTEPLIPFAPFVRVVKELTGFITDWRIGRYTPEALLALQEAAEFHLIELFQVANLCAIHAKRVTVMQKDIQLARRIGGKRWAYPFFLPY

SEQ ID NO: 94 - protein, 97 aa, Artificial Sequence
  Brassica napa turnip CENH3 histone domain
PGTVALREIRHFQKTTKLLIPAASFIREVRSVTQIFAPPDVTRWTAEALMAIQEAAEDFLVGLFSDAMLCAIHARRVTLMRKDFELARRLGGKGRPL

SEQ ID NO: 95 - protein, 43 aa, Artificial Sequence
  conserved plant tail domain of H3 histone protein, N-terminal tail of H3, H3 tail
MARTKQSARKSHGGKAPTKQLATKAARKSAPTTGGVKKPHRFR

SEQ ID NO: 96 - protein, 705 aa, Arabidopsis thaliana
  thale cress centromere protein C (CENPC)
MADVSRSSSLYTEEDPLQAYSGLSLFPRTLKSLSNPLPPSYQSEDLQQTHTLLQSMPFEIQSEHQEQAKAILEDVDVDVQLNPIPNKRERRPGLDRKRKSFSLHLTTSQPPPVAPSFDPSKYPRSEDFFAAYDKFELANREWQKQTGSSVIDIQENPPSRRPRRPGIPGRKRRPFKESFTDSYFTDVINLEASEKEIPIASEQSLESATAAHVTTVDREVDDSTVDTDKDLNNVLKDLLACSREELEGDGAIKLLEERLQIKSFNIEKFSIPEFQDVRKMNLKASGSNPPNRKSLSDIQNILKGTNRVAVRKNSHSPSPQTIKHFSSPNPPVDQFSFPDIHNLLPGDQQPSEVNVQPIAKDIPNTSPTNVGTVDVASPFNDSVVKRSGEDDSHIHSGIHRSHLSRDGNPDICVMDSISNRSSAMLQKNVDMRTKGKEVDVPMSESGANRNTGDRENDAEINEETDNLERLAECASKEVTRPFTVEEDSIPYQQGASSKSPNRAPEQYNTMGGSLEHAEHNQGLHEEENVNTGSASGLQVENAPEVHKYSHKQTNKRRKRGSSDSNVKKRSKTVHGETGGDKQMKTLPHESRAKKQTKGKSNEREEKKPKKTLTHEGKLFSCRKSLAAAGTKIEGGVRRSTRIKSRPLEYWRGERFLYGRIHESLTTVIGIKYASPGEGKRDSRASKVKSFVSDEYKKLVDFAALH

SEQ ID NO: 97 - protein, 312 aa, Arabidopsis thaliana
  thale cress MCM21
MGEMIVSMDQDIRLDTTRARLSNLLKRHRELSDRLTRDSDKTMLDRLNKEFEAARRSQSQEVFLDGEEWNDGLLATLRERVHMEADRKADNGNAGFSLVCHPEERITYRVGNKVICCLDGSRIGIQFETSTAGETYEVYHCVLESKSFLEKMIVLEHTIPFFLPLSDLENDLLFSNAKKFIDNVGDLLQAYVDRKEQVRLIKELFGHQISEIYHSLPYHMIEFSMDDCDCKFVVSLRYGDLLCELPTKVRILVWPMHHLSKKQCTSPGSPAIPVRLPFAEDAFRIQSLPEAYAEIMPNMPNEIRQLFQTSPS

SEQ ID NO: 98 - protein, 285 aa, Arabidopsis thaliana
  thale cress minichromosome instability 12 (MIS12)
MEGSKSEAVFDSMNLNPQIFINEAINSVEDYVDQAFDFYARDASKSLKIKGSDKQKSQALSNGIARVRGLLLSVIDNRLKLWESYSLRFCFAVPDGFVLPKSEESSSVHQDGLYDLELDAELDSLRDKLNVVGKRSVELDSELQALERSSVSRERSLRLVNEALELYDESSMDEIFKEMTKMASELRASVERLKTRRMKASESAKVKRLKNHGKEFSAMTFDYVVSGLPNGGSRQKPVIPPDQKPQHIILVSSQVSLELATSKLRLGSLPIELTTLDYFCMCFIM

SEQ ID NO: 99 - protein, 568 aa, Arabidopsis thaliana
  thale cress NDC80
MRGGAAGKRRTTVGFGGAPPPPPPSIEQQRHLFNSRDSDASFASSRPSSIGLGGRGASDDRSSMIRFINAFLSTHNFPISIRGNPVPSVKDISETLKFLLSALDYPCDSIKWDEDLVFFLKSQKCPFKITKSSLKAPNTPHNWPTVLAVVHWLAELARFHQHLVSNSTSVPEDNSMNFFAIQSFGHFIRGEDDKVNDLDSQFLGKLEAEKTSVAETISGCEKISGELEAKLESLRKGPSKKESLEKVKADLENDVNKFRTIVVEYTDRNPAMEKVVEEKAKELKAKEEERERISVENKELKKSVELQNFSAADVNRMRRELQAVERDVADAEVARDGWDQKAWELNSQIRNQFHQIQTLAIDCNQALRRLKLDIQFAVNERGETPAAVMGVDYKSVVKPALCSLCDGIKGSSAEKVEELVTLQHHKSEMASKIESKRSLLGSIQLQINDLEEKMKLVKKETQELSTKCDLEAKTLVESVKAEALNLEVVEKEAAEFVKASELRLQEAVKESEEEVQACAAQLFALIDSISKQKEYMDSKISEIKTGVADTASAVSEIYKANFKKNLGI

SEQ ID NO: 100 - protein, 440 aa, Arabidopsis thaliana
  thale cress NUF2
MSAYEYPRLSRSDIITALKDAQIASVTETDLKTPTSDFVSELYTRILIYLDALDEEEKGQVDFEALEQLENPDHHATSMQAMKLYCKVKDMLEMLDCPLPISFKDLLRPESSRTEFFISALLNYGLYKDSKMDLIRPKAEELGLLDEQRKQCEAKVAQLNAEIGEFDEAVERDLPFVQELEANIEQLNKKILELNNQQMSLRATFQKMREKSTQMDNEISKAEFDLVETVQENANLRSQIVQSPDKLQGALEEKKLVLGETKKAEQSAMVTFQEKAAILEVFEKALKKILKSSSQLQLINEQVTNAKTVEKEFKALKDKLSEDGVAYKSLEAKVVERERIVEQLNESLKQLEKEKAVMFDDWTKQLNELKVEVESRRRELETRQTNVESVVAMVDDNTAKTNQVRQSGEAKVKKLAAKYEEIVKQFHEYTVSFDAFLPSL

SEQ ID NO: 101 - DNA, 1109 bp, Artificial Sequence
  synthetic maize CENH3 tail, Arabidopsis histone-fold domain
atggctcgaaccaagcaccaggccgtgaggaagacggcggagaagcccaagaagaagctccagttcgagcgctcaggtggtgcgagtacctcggcgacgccggaaagggctgctgggaccgggggaagagcggcgtctggaggtgactcagttaagaagacgaaaccacgccaccgctggaggccaggaaccgttgctctaaaagagattcgccatttccagaagcagacaaaccttcttattccggctgccagtttcataagagaagttagttactctttttcttaccagccataataagtttcacagcttaacaatattcatatatactaacagaggcacaagccttttggtgtttaatgtggctagttttaggatttgcacaccccacacatatctgagcatcaatgcagtgtacatagtgagtgatatagcaatttaactaaaattcagagtaatcgtgaggccaaccctccttgtttaaggagtgtgtaatctagtttgtctttgaggttatgagctcatagattcagaaccatatgattcctgtagctacaaaactcaacatgaatcgtcagtgatgtggaaatgctgatttgtgttacaaacaaactattttacattgtttttccaggtgagaagtataacccatatgttggcccctccccaaatcaatcgttggacagctgaagctcttgttgctcttcaagaggtaccaatccttcaactttttctttatacgaatgtatgaatatagatatagagatagtcacacatttcaactaatgtcattccccttgatgaccaatcaacctaatcacacaaattctttgtggtaggcggcagaagattacttggttggtttgttctcagattcaatgctctgtgctatccatgcaagacgtgttactctaagtaagtactctaaaagaagacatttttcagtctcaacttaggaatcacaagcatacattttatatccctttgaatcattagttacttgaatatcatatataaaaatgcttatctatatctgttttttgttcatatcagtgagaaaagactttgaacttgcacgccggcttggaggaaaaggcagaccatggtga

SEQ ID NO: 102 - DNA, 477 bp, Artificial Sequence
  synthetic maize CENH3 tail cDNA
atggctcgaaccaagcaccaggccgtgaggaagacggcggagaagcccaagaagaagctccagttcgagcgctcaggtggtgcgagtacctcggcgacgccggaaagggctgctgggaccgggggaagagcggcgtctggaggtgactcagttaagaagacgaaaccacgccaccgctggaggccaggaaccgttgctctaaaagagattcgccatttccagaagcagacaaaccttcttattccggctgccagtttcataagagaagtgagaagtataacccatatgttggcccctccccaaatcaatcgttggacagctgaagctcttgttgctcttcaagaggcggcagaagattacttggttggtttgttctcagattcaatgctctgtgctatccatgcaagacgtgttactctaatgagaaaagactttgaacttgcacgccggcttggaggaaaaggcagaccatggtga

SEQ ID NO: 103 - protein, 158 aa, Artificial Sequence
  synthetic maize tailswap protein
MARTKHQAVRKTAEKPKKKLQFERSGGASTSATPERAAGTGGRAASGGDSVKKTKPRHRWRPGTVALKEIRHFQKQTNLLIPAASFIREVRSITHMLAPPQINRWTAEALVALQEAAEDYLVGLFSDSMLCAIHARRVTLMRKDFELARRLGGKGRPW

SEQ ID NO: 104 - DNA, 708 bp, Artificial Sequence
  synthetic mCherry red fluorescent protein DsRed variant
atggtgagcaagggcgaggaggataacatggccatcatcaaggagttcatgcgcttcaaggtgcacatggagggctccgtgaacggccacgagttcgagatcgagggcgagggcgagggccgcccctacgagggcacccagaccgccaagctgaaggtgaccaagggtggccccctgcccttcgcctgggacatcctgtcccctcagttcatgtacggctccaaggcctacgtgaagcaccccgccgacatccccgactacttgaagctgtccttccccgagggcttcaagtgggagcgcgtgatgaacttcgaggacggcggcgtggtgaccgtgacccaggactcctccctgcaggacggcgagttcatctacaaggtgaagctgcgcggcaccaacttcccctccgacggccccgtaatgcagaagaagaccatgggctgggaggcctcctccgagcggatgtaccccgaggacggcgccctgaagggcgagatcaagcagaggctgaagctgaaggacggcggccactacgacgctgaggtcaagaccacctacaaggccaagaagcccgtgcagctgcccggcgcctacaacgtcaacatcaagttggacatcacctcccacaacgaggactacaccatcgtggaacagtacgaacgcgccgagggccgccactccaccggcggcatggacgagctgtacaag

SEQ ID NO: 105 - protein, 236 aa, Artificial Sequence
  synthetic mCherry red fluorescent protein DsRed variant
MVSKGEEDNMAIIKEFMRFKVHMEGSVNGHEFEIEGEGEGRPYEGTQTAKLKVTKGGPLPFAWDILSPQFMYGSKAYVKHPADIPDYLKLSFPEGFKWERVMNFEDGGVVTVTQDSSLQDGEFIYKVKLRGTNFPSDGPVMQKKTMGWEASSERMYPEDGALKGEIKQRLKLKDGGHYDAEVKTTYKAKKPVQLPGAYNVNIKLDITSHNEDYTIVEQYERAEGRHSTGGMDELYK

SEQ ID NO: 106 - protein, 211 aa, Candida albicans
  yeast CENH3
MARLSGQSSGRQTGQGTSAEAIRQQREELRRQRELRLQQQQQAERQQQRQQYRTEQSPIVPAATSSSRYSQFGIYRNQPGDVVDTLASSLPRRTTTTRPEVNRTVPRVKKRYRPGTKALREIRQYQKSTDLLIRKLPFARLVREISLDFVGPSYGLRWQSNAILALQEASESFLIHLLEDTNLCAIHAKRVTIMQKDIQLARRIRGQSWIL

SEQ ID NO: 107 - protein, 140 aa, Homo sapiens
  human CENH3
MGPRRRSRKPEAPRRRSPSPTPTPGPSRRGPSLGASSHQHSRRRQGWLKEIRKLQKSTHLLIRKLPFSRLAREICVKFTRGVDFNWQAQALLALQEAAEAFLVHLFEDAYLLTLHAGRVTLFPKDVQLARRIRGLEEGLG

SEQ ID NO: 108 - protein, 164 aa, Oryza sativa
  rice centromeric histone 3 (CENH3)
MARTKHPAVRKSKAEPKKKLQFERSPRPSKAQRAGGGTGTSATTRSAAGTSASGTPRQQTKQRKPHRFRPGTVALREIRKFQKTTELLIPFAPFSRLVREITDFYSKDVSRWTLEALLALQEAAEYHLVDIFEVSNLCAIHAKRVTIMQKDMQLARRIGGRRPW

SEQ ID NO: 109 - protein, 97 aa, Artificial Sequence; identical to SEQ ID NO: 56
  synthetic CENH3 histone-fold domain

SEQ ID NO: 110 - DNA, 30 bp, Artificial Sequence
  synthetic PCR amplification primer CP 384
  modified_base (1)...(4): n = g, a, c or t
nnnngtcgacatggctcgaaccaagcacca

SEQ ID NO: 111 - DNA, 27 bp, Artificial Sequence
  synthetic PCR amplification primer CP 572
caacggttcctggcctccagcggtggc

SEQ ID NO: 112 - DNA, 27 bp, Artificial Sequence
  synthetic PCR amplification primer CP 571
gccaccgctggaggccaggaaccgttg

SEQ ID NO: 113 - DNA, 34 bp, Artificial Sequence
  synthetic PCR amplification primer CP 375
  modified_base (1)...(4): n = g, a, c or t
nnnntctagatcaccatggtctgccttttcctcc

SEQ ID NO: 114 - protein, 6 aa, Artificial Sequence
  synthetic conserved sequence at border between tail domain and histone-fold domain of CENH3 proteins
PGTVAL